European Patent Application EP 4 678 655 A1, published January 14, 2026. Title: 조절 T 세포 표면 항원의 에피토프 및 이에 특이적으로 결합하는 항체. Applicant: 주식회사 굳티셀. The sequence listing filed with the application follows.

SEQUENCE LISTING (69 sequences)

SEQ ID NO: 1 - protein, 1093 aa, Homo sapiens [sequence omitted]

SEQ ID NO: 2 - DNA, 3282 bp, Homo sapiens
  source 1..3282: mol_type = genomic DNA
atggcgcggccggtccggggagggctcggggccccgcgccgctcgccttgccttctccttctctggctgcttttgcttcggctggagccggtgaccgccgcggccggcccgcgggcgccctgcgcggccgcctgcacttgcgctggggactcgctggactgcggtgggcgcgggctggctgcgttgcccggggacctgccctcctggacgcggagcctaaacctgagttacaacaaactctctgagattgaccctgctggttttgaggacttgccgaacctacaggaagtgtacctcaataataatgagttgacagcggtaccatccctgggcgctgcttcatcacatgtcgtctctctctttctgcagcacaacaagattcgcagcgtggaggggagccagctgaaggcctacctttccttagaagtgttagatctgagtttgaacaacatcacggaagtgcggaacacctgctttccacacggaccgcctataaaggagctcaacctggcaggcaatcggattggcaccctggagttgggagcatttgatggtctgtcacggtcgctgctaactcttcgcctgagcaaaaacaggatcacccagcttcctgtaagagcattcaagctacccaggctgacacaactggacctcaatcggaacaggattcggctgatagagggcctcaccttccaggggctcaacagcttggaggtgctgaagcttcagcgaaacaacatcagcaaactgacagatggggccttctggggactgtccaagatgcatgtgctgcacctggagtacaacagcctggtagaagtgaacagcggctcgctctacggcctcacggccctgcatcagctccacctcagcaacaattccatcgctcgcattcaccgcaagggctggagcttctgccagaagctgcatgagttggtcctgtccttcaacaacctgacacggctggacgaggagagcctggccgagctgagcagcctgagtgtcctgcgtctcagccacaattccatcagccacattgcggagggtgccttcaagggactcaggagcctgcgagtcttggatctggaccataacgagatttcgggcacaatagaggacacgagcggcgccttctcagggctcgacagcctcagcaagctgactctgtttggaaacaagatcaagtctgtggctaagagagcattctcggggctggaaggcctggagcacctgaaccttggagggaatgcgatcagatctgtccagtttgatgcctttgtgaagatgaagaatcttaaagagctccatatcagcagcgacagcttcctgtgtgactgccagctgaagtggctgcccccgtggctaattggcaggatgctgcaggcctttgtgacagccacctgtgcccacccagaatcactgaagggtcagagcattttctctgtgccaccagagagtttcgtgtgcgatgacttcctgaagccacagatcatcacccagccagaaaccaccatggctatggtgggcaaggacatccggtttacatgctcagcagccagcagcagcagctcccccatgacctttgcctggaagaaagacaatgaagtcctgaccaatgcagacatggagaactttgtccacgtccacgcgcaggacggggaagtgatggagtacaccaccatcctgcacctccgtcaggtcactttcgggcacgagggccgctaccaatgtgtcatcaccaaccactttggctccacctattcacataaggccaggctcaccgtgaatgtgttgccatcattcaccaaaacgccccacgacataaccatccggaccaccaccatggcccgcctcgaatgtgctgccacaggtcacccaaaccctcagattgcctggcagaaggatggaggcacggatttccccgctgcccgtgagcgacgcatgcatgtcatgccggatgacgacgtgtttttcatcactgatgtgaaaatagatgacgcaggggtttacagctgtactgctcagaactcagccggttctatttcagctaatgccaccctgactgtcctagagaccccatccttggtggtccccttggaagaccgtgtggtatctgtgggagaaacagtggccctccaatgcaaagccacggggaaccctccgccccgcatcacctggttcaagggggaccgcccgctgagcctcactgagcggcaccacttgacccctgacaaccagctcctggtggttcagaacgtggtggcagaggatgcgggccgatatacctgtgagatgtccaacaccctgggcacggagcgagctcacagccagctgagcgtcctgcccgcagcaggctgcaggaaggatgggaccacggtaggcatcttcaccattgctgtcgtgagcagcatcgtcctgacgtcactggtctgggtgtgcatcatctaccagaccaggaagaagagtgaagagtacagtgtcaccaacacagatgaaaccgtcgtgccaccagatgttccaagctacctctcttctcaggggaccctttctgaccgacaagaaaccgtggtcaggaccgagggtggccctcaggccaatgggcacattgagagcaatggtgtgtgtccaagagatgcaagccactttccagagcccgacactcacagcgttgcctgcaggcagccaaagctctgtgctgggtctgcgtatcacaaagagccgtggaaagcgatggagaaagctgaagggacacctgggccacataagatggaacacggtggccgggtcgtatgcagtgactgcaacaccgaagtggactgttactccaggggacaagccttccacccccagcctgtgtccagagacagcgcacagccaagtgcgccaaatggcccggagccgggtgggagtgaccaagagcattctccacatcaccagtgcagcaggactgccgctgggtcctgccccgagtgccaagggtcgctctaccccagtaaccacgatagaatgctgacggctgtgaagaaaaagccaatggcatctctagatgggaaaggggattcttcctggactttagcaaggttgtatcacccggactccacagagctacagcctgcatcttcattaacttcaggcagtccagagcgcgcggaagcccagtacttgcttgtttccaatggccacctccccaaagcatgtgacgccagtcccgagtccacgccactgacaggacagctccccgggaaacagagggtgccactgctgttggcaccaaaaagctag

SEQ ID NO: 3 - protein, 1091 aa, Mus musculus
MARPGPGVLGAPRLAPRLLLWLLLLLLQWPESAGAQAGPRAPCAAACTCAGDSLDCSGRGLATLPRDLPSWTRSLNLSYNRLSEIDSAAFEDLTNLQEVYLNSNELTAIPSLGTASIGVVSLFLQHNKILSVDGSQLKSYLSLEVLDLSSNNITEIRSSCFPNGLRIRELNLASNRISILESGAFDGLSRSLLTLRLSKNRITQLPVKAFKLPRLTQLDLNRNRIRLIEGLTFQGLDSLEVLRLQRNNISRLTDGAFWGLSKMHVLHLEYNSLVEVNSGSLYGLTALHQLHLSNNSISRIQRDGWSFCQKLHELILSFNNLTRLDEESLAELSSLSILRLSHNAISHIAEGAFKGLKSLRVLDLDHNEISGTIEDTSGAFTGLDNLSKLTLFGNKIKSVAKRAFSGLESLEHLNLGENAIRSVQFDAFAKMKNLKELYISSESFLCDCQLKWLPPWLMGRMLQAFVTATCAHPESLKGQSIFSVLPDSFVCDDFPKPQIITQPETTMAVVGKDIRFTCSAASSSSSPMTFAWKKDNEVLANADMENFAHVRAQDGEVMEYTTILHLRHVTFGHEGRYQCIITNHFGSTYSHKARLTVNVLPSFTKIPHDIAIRTGTTARLECAATGHPNPQIAWQKDGGTDFPAARERRMHVMPDDDVFFITDVKIDDMGVYSCTAQNSAGSVSANATLTVLETPSLAVPLEDRVVTVGETVAFQCKATGSPTPRITWLKGGRPLSLTERHHFTPGNQLLVVQNVMIDDAGRYTCEMSNPLGTERAHSQLSILPTPGCRKDGTTVGIFTIAVVCSIVLTSLVWVCIIYQTRKKSEEYSVTNTDETIVPPDVPSYLSSQGTLSDRQETVVRTEGGHQANGHIESNGVCLRDPSLFPEVDIHSTTCRQPKLCVGYTREPWKVTEKADRTAAPHTTAHSGSAVCSDCSTDTAYHPQPVPRDSGQPGTASSQELRQHDREYSPHHPYSGTADGSHTLSGGSLYPSNHDRILPSLKNKAASADGNGDSSWTLAKLHEADCIDLKPSPTLASGSPELMEDAISTEAQHLLVSNGHLPKACDSSPESVPLKGQITGKRRGPLLLAPRS

SEQ ID NO: 4 - DNA, 3276 bp, Mus musculus
  source 1..3276: mol_type = genomic DNA
atggcgcggcccggtccgggagtgctcggagccccgcgccttgcgcctcgccttctgctctggctgctcttgctgctactgcaatggccggagtcagcgggcgcccaggctcgcccgcgggccccctgcgcggccgcctgcacttgcgccgggaactcgctggactgcagtgggcgcgggctggcgacgctgccccgggacctgccctcctggacgcgcagcctaaacctgagttataacagactctccgagatcgactctgctgcttttgaggacttgacgaatctgcaggaagtgtacctcaacagcaatgagctgacagccataccatcactgggcactgcttccataggagttgtctctctctttttgcagcacaacaagatccttagtgtggatgggagccagctgaagtcgtacctgtccttggaagtgctggatctgagttccaacaacatcacggaaattcggagctcctgtttcccgaacggcctgcgtataagggaactcaacttggcgagcaaccgcatcagcatcctggagtctggagcatttgatggtctgtcgcggtcactgctgactctccgtctgagcaaaaacaggatcacccagcttcctgtgaaagcgttcaagctacccaggctgacacaactagacctgaatcggaatcggattcggctgattgaaggcctcacgttccaggggctcgacagcttagaggtgctgaggcttcagaggaacaacatcagcaggctgacggacggggccttctgggggctgtctaagatgcacgtgctgcacctggagtacaacagtctggtggaagtgaacagtggctccctctatggcctcacagccctgcaccagctgcacctcagcaacaactccatctctcgaattcagcgtgatggctggagcttctgccaaaagctgcatgagttgattctgtccttcaacaacctcacgcggctggatgaggagagtctagcggagttgagcagcctcagtatcctgcgcctcagtcacaacgccatcagtcacattgctgaaggcgccttcaagggactcaagagtctgcgggtcttggacctggaccataacgagatctcgggtacaatcgaggataccagtggtgcctttacggggcttgacaacctcagcaagctgactctgtttggaaacaagatcaaatctgtggctaagagagccttctcgggcctggaaagcctggaacacctgaaccttggagagaatgcaatcaggtctgtccagtttgatgcctttgcaaagatgaagaaccttaaagagctctacatcagcagtgagagcttcctgtgtgactgccagctcaagtggctgcccccatggctaatgggtaggatgctgcaggcctttgtgacagccacctgtgcccatccagagtcgctgaagggccagagcattttctcagtgctgccagacagctttgtgtgtgatgactttccaaagccacagatcatcacccagcctgagacgaccatggctgtggtgggcaaggacatccgtttcacatgctccgcagccagcagcagcagctcaccaatgaccttcgcctggaagaaggacaatgaggtcctggccaatgcagacatggagaactttgcccacgtccgtgcacaggacggcgaagtgatggagtataccactatcctgcacctccgtcacgtcacctttgggcacgagggccgctaccagtgtatcatcacaaaccactttggctccacatactcccacaaagccaggctcactgtgaatgtgttgccatcattcactaaaataccccatgacattgccatccggactggcaccacagcccgcctcgagtgtgctgccacgggccaccctaaccctcagattgcctggcagaaggatggaggcaccgatttcccggcagctcgtgagcgacgcatgcatgttatgccagacgatgatgtgttcttcatcactgatgtgaaaatagacgacatgggggtctacagctgcactgcccagaactcggcaggctcggtttcagccaacgctaccctcacagtcttagaaactccatccttggcagtgcctctggaagaccgtgtggtaactgtgggagaaacagtggccttccagtgcaaagcaaccgggagccccacaccacgcatcacctggcttaagggaggtcgcccattgagcctcacagagcgccaccatttcactccaggcaaccagctgctggttgttcagaatgtgatgatagacgatgcagggcggtatacctgtgagatgtctaatcccctgggcactgagcgagcacatagccagctgagcattttacctacccctggctgccggaaggatgggaccaccgtaggcatcttcaccattgctgtggtgtgcagtattgtcctgacctcgctggtgtgggtgtgcatcatctaccagaccaggaagaagagcgaggagtacagcgtcactaacacagatgaaaccattgtgcctccagatgttccaagctacctctcctctcagggaaccctttctgaccggcaggaaactgtggtcaggactgagggtggtcatcaggccaatgggcacattgaaagcaatggtgtgtgtctgagagacccgagcctcttcccagaggtcgacattcatagcactacatgtaggcagcccaagctgtgtgttggatacactagagagccctggaaggtgacggagaaagccgacaggacagctgccccacatacaacagcacacagtggctctgctgtatgtagtgactgcagtactgacacagcctaccatccccagcctgtgcccagagacagtgggcagccaggcacagcgagcagccaagagctcaggcagcatgaccgggaatattctccacaccatccttacagtgggactgcggatgggtctcataccctctctggggggtccctctatccaagcaaccatgacagaatactgccatccttgaagaacaaggcggcgtctgcagatgggaacggagattcctcttggactttagcaaagttacatgaagcagactgcatagacctaaagccttctcctacgttagcttcaggcagcccagagctcatggaagacgccatatctactgaagcccagcacttgcttgtttccaatggccacctccccaaggcctgtgactccagccctgaatctgtgccactgaaagggcagatcactgggaaacggaggggaccactgctattggcaccgagaagctag

SEQ ID NO: 5 - protein, 764 aa, Homo sapiens
AGPRAPCAAACTCAGDSLDCGGRGLAALPGDLPSWTRSLNLSYNKLSEIDPAGFEDLPNLQEVYLNNNELTAVPSLGAASSHVVSLFLQHNKIRSVEGSQLKAYLSLEVLDLSLNNITEVRNTCFPHGPPIKELNLAGNRIGTLELGAFDGLSRSLLTLRLSKNRITQLPVRAFKLPRLTQLDLNRNRIRLIEGLTFQGLNSLEVLKLQRNNISKLTDGAFWGLSKMHVLHLEYNSLVEVNSGSLYGLTALHQLHLSNNSIARIHRKGWSFCQKLHELVLSFNNLTRLDEESLAELSSLSVLRLSHNSISHIAEGAFKGLRSLRVLDLDHNEISGTIEDTSGAFSGLDSLSKLTLFGNKIKSVAKRAFSGLEGLEHLNLGGNAIRSVQFDAFVKMKNLKELHISSDSFLCDCQLKWLPPWLIGRMLQAFVTATCAHPESLKGQSIFSVPPESFVCDDFLKPQIITQPETTMAMVGKDIRFTCSAASSSSSPMTFAWKKDNEVLTNADMENFVHVHAQDGEVMEYTTILHLRQVTFGHEGRYQCVITNHFGSTYSHKARLTVNVLPSFTKTPHDITIRTTTVARLECAATGHPNPQIAWQKDGGTDFPAARERRMHVMPDDDVFFITDVKIDDAGVYSCTAQNSAGSISANATLTVLETPSLVVPLEDRVVSVGETVALQCKATGNPPPRITWFKGDRPLSLTERHHLTPDNQLLVVQNVVAEDAGRYTCEMSNTLGTERAHSQLSVLPAAGCRKDGTTHHHHHH

SEQ ID NO: 6 - protein, 760 aa, Mus musculus
AQAGPRAPCAAACTCAGDSLDCSGRGLATLPRDLPSWTRSLNLSYNRLSEIDSAAFEDLTNLQEVYLNSNELTAIPSLGAASIGVVSLFLQHNKILSVDGSQLKSYLSLEVLDLSSNNITEIRSSCFPNGLRIRELNLASNRISILESGAFDGLSRSLLTLRLSKNRITQLPVKAFKLPRLTQLDLNRNRIRLIEGLTFQGLDSLEVLRLQRNNISRLTDGAFWGLSKMHVLHLEYNSLVEVNSGSLYGLTALHQLHLSNNSISRIQRDGWSFCQKLHELILSFNNLTRLDEESLAELSSLSILRLSHNAISHIAEGAFKGLKSLRVLDLDHNEISGTIEDTSGAFTGLDNLSKLTLFGNKIKSVAKRAFSGLESLEHLNLGENAIRSVQFDAFAKMKNLKELYISSESFLCDCQLKWLPPWLMGRMLQAFVTATCAHPESLKGQSIFSVLPDSFVCDDFPKPQIITQPETTMAVVGKDIRFTCSAASSSSSPMTFAWKKDNEVLANADMENFAHVRAQDGEVMEYTTILHLRHVTFGHEGRYQCIITNHFGSTYSHKARLTVNVLPSFTKIPHDIAIRTGTTARLECAATGHPNPQIAWQKDGGTDFPAARERRMHVMPDDDVFFITDVKIDDMGVYSCTAQNSAGSVSANATLTVLETPSLAVPLEDRVVTVGETVAFQCKATGSPTPRITWLKGGRPLSLTERHHFTPGNQLLVVQNVMIDDAGRYTCEMSNPLGTERAHSQLSILPTPGCRKDGTT

SEQ ID NO: 7 - protein, 5 aa, synthetic construct
NYAMS

SEQ ID NO: 8 - protein, 17 aa, synthetic construct
VISHGGGSTYYADSVKG

SEQ ID NO: 9 - protein, 18 aa, synthetic construct
VISNCHLGVCYYSNGMDV

SEQ ID NO: 10 - protein, 13 aa, synthetic construct
SGSSSNIGDNYVS

SEQ ID NO: 11 - protein, 7 aa, synthetic construct
DNNKRPS

SEQ ID NO: 12 - protein, 10 aa, synthetic construct
WDGSLSAGRV

SEQ ID NO: 13 - protein, 127 aa, synthetic construct
EVQLLESGGGLVQPGGSLRLSCAASGFTFSNYAMSWVRQAPGKGLEWVSVISHGGGSTYYADSVKGRFTISRDNSKNTLYLQMNSLRAEDTAVYYCARVISNCHLGVCYYSNGMDVWGQGTLVTVSS

SEQ ID NO: 14 - protein, 111 aa, synthetic construct
QLVLTQPPSVSAAPGQRVSISCSGSSSNIGDNYVSWYQQVPGSAPKLLIYDNNKRPSGIPDRFSASKSGTSATLGITGLQTGDEADYYCATWDGSLSAGRVFGGGTKLTVL

SEQ ID NO: 15 - protein, 457 aa, synthetic construct
EVQLLESGGGLVQPGGSLRLSCAASGFTFSNYAMSWVRQAPGKGLEWVSVISHGGGSTYYADSVKGRFTISRDNSKNTLYLQMNSLRAEDTAVYYCARVISNCHLGVCYYSNGMDVWGQGTLVTVSSAKTTAPSVYPLAPVCGDTTGSSVTLGCLVKGYFPEPVTLTWNSGSLSSGVHTFPAVLQSDLYTLSSSVTVTSSTWPSQSITCNVAHPASSTKVDKKIEPRGPTIKPCPPCKCPAPNLLGGPSVFIFPPKIKDVLMISLSPIVTCVVVDVSEDDPDVQISWFVNNVEVHTAQTQTHREDYNSTLRVVSALPIQHQDWMSGKEFKCKVNNKDLPAPIERTISKPKGSVRAPQVYVLPPPEEEMTKKQVTLTCMVTDFMPEDIYVEWTNNGKTELNYKNTEPVLDSDGSYFMYSKLRVEKKNWVERNSYSCSVVHEGLHNHHTTKSFSRTPGK

SEQ ID NO: 16 - protein, 218 aa, synthetic construct
QLVLTQPPSVSAAPGQRVSISCSGSSSNIGDNYVSWYQQVPGSAPKLLIYDNNKRPSGIPDRFSASKSGTSATLGITGLQTGDEADYYCATWDGSLSAGRVFGGGTKLTVLRADAAPTVSIFPPSSEQLTSGGASVVCFLNNFYPKDINVKWKIDGSERQNGVLNSWTDQDSKDSTYSMSSTLTLTKDEYERHNSYTCEATHKTSTSPIVKSFNRNEC

SEQ ID NO: 17 - protein, 457 aa, synthetic construct
EVQLLESGGGLVQPGGSLRLSCAASGFTFSNYAMSWVRQAPGKGLEWVSVISHGGGSTYYADSVKGRFTISRDNSKNTLYLQMNSLRAEDTAVYYCARVISNCHLGVCYYSNGMDVWGQGTLVTVSSASTKGPSVFPLAPSSKSTSGGTAALGCLVKDYFPEPVTVSWNSGALTSGVHTFPAVLQSSGLYSLSSVVTVPSSSLGTQTYICNVNHKPSNTKVDKKVEPKSCDKTHTCPPCPAPELLGGPSVFLFPPKPKDTLMISRTPEVTCVVVDVSHEDPEVKFNWYVDGVEVHNAKTKPREEQYNSTYRVVSVLTVLHQDWLNGKEYKCKVSNKALPAPIEKTISKAKGQPREPQVYTLPPSREEMTKNQVSLTCLVKGFYPSDIAVEWESNGQPENNYKTTPPVLDSDGSFFLYSKLTVDKSRWQQGNVFSCSVMHEALHNHYTQKSLSLSPGK

SEQ ID NO: 18 - protein, 218 aa, synthetic construct
QLVLTQPPSVSAAPGQRVSISCSGSSSNIGDNYVSWYQQVPGSAPKLLIYDNNKRPSGIPDRFSASKSGTSATLGITGLQTGDEADYYCATWDGSLSAGRVFGGGTKLTVLRTVAAPSVFIFPPSDEQLKSGTASVVCLLNNFYPREAKVQWKVDNALQSGNSQESVTEQDSKDSTYSLSSTLTLSKADYEKHKVYACEVTHQGLSSPVTKSFNRGEC

SEQ ID NO: 19 - protein, 455 aa, synthetic construct
EVQLLESGGGLVQPGGSLRLSCAASGFTFSNYAMSWVRQAPGKGLEWVSVISHGGGSTYYADSVKGRFTISRDNSKNTLYLQMNSLRAEDTAVYYCARVISNCHLGVCYYSNGMDVWGQGTLVTVSSTTAPSVYPLAPVCGDTTGSSVTLGCLVKGYFPEPVTLTWNSGSLSSGVHTFPAVLQSDLYTLSSSVTVTSSTWPSQSITCNVAHPASSTKVDKKIEPRGPTIKPCPPCKCPAPNLLGGPSVFIFPPKIKDVLMISLSPIVTCVVVDVSEDDPDVQISWFVNNVEVHTAQTQTHREDYNSTLRVVSALPIQHQDWMSGKEFKCKVNNKDLPAPIERTISKPKGSVRAPQVYVLPPPEEEMTKKQVTLTCMVTDFMPEDIYVEWTNNGKTELNYKNTEPVLDSDGSYFMYSKLRVEKKNWVERNSYSCSVVHEGLHNHHTTKSFSRTPGK

SEQ ID NO: 20 - protein, 217 aa, synthetic construct
QSVLTQPPSASGTPGQRVTISCSGSSSNIGNNDVYWYQQLPGTAPKLLIYSDSQRPSGVPDRFSGSKSGTSASLAISGLRSEDEADYYCGTWDYSLSGYVFGGGTKLTVLRTVAAPTVSIFPPSSEQLTSGGASVVCFLNNFYPKDINVKWKIDGSERQNGVLNSWTDQDSKDSTYSMSSTLTLTKDEYERHNSYTCEATHKTSTSPIVKSFNRNEC

SEQ ID NO: 21 - protein, 22 aa, synthetic construct
DIRFTCSAASSSSSPMTFAWKK

SEQ ID NO: 22 - protein, 19 aa, synthetic construct
FTCSAASSSSSPMTFAWKK

SEQ ID NO: 23 - protein, 52 aa, synthetic construct
FTCSAASSSSSPMTFAWKKDNEVLTNADMENFVHVHAQDGEVMEYTTILHLR

SEQ ID NO: 24 - protein, 27 aa, synthetic construct
QVTFGHEGRYQCVITNHFGSTYSHKAR

SEQ ID NO: 25 - protein, 18 aa, synthetic construct
YQCVITNHFGSTYSHKAR

SEQ ID NO: 26 - protein, 30 aa, synthetic construct
AWKKDNEVLTNADMENFVHVHAQDGEVMEY

SEQ ID NO: 27 - protein, 31 aa, synthetic construct
FAWKKDNEVLTNADMENFVHVHAQDGEVMEY

SEQ ID NO: 28 - protein, 10 aa, synthetic construct
KKDNEVLTNA

SEQ ID NO: 29 - protein, 28 aa, synthetic construct
KKDNEVLTNADMENFVHVHAQDGEVMEY

SEQ ID NO: 30 - protein, 9 aa, synthetic construct
VHAQDGEVM

SEQ ID NO: 31 - protein, 82 aa, synthetic construct
DIRFTCSAASSSSSPMTFAWKKDNEVLTNADMENFVHVHAQDGEVMEYTTILHLRQVTFGHEGRYQCVITNHFGSTYSHKAR

SEQ ID NO: 32 - protein, 38 aa, synthetic construct
AYLSLEVLDLSLNNITEVRNTCFPHGPPIKELNLAGNR

SEQ ID NO: 33 - protein, 9 aa, synthetic construct
NRITQLPVR

SEQ ID NO: 34 - protein, 48 aa, synthetic construct
LTDGAFWGLSKMHVLHLEYNSLVEVNSGSLYGLTALHQLHLSNNSIAR

SEQ ID NO: 35 - protein, 37 aa, synthetic construct
KGWSFCQKLHELVLSFNNLTRLDEESLAELSSLSVLR

SEQ ID NO: 36 - protein, 20 aa, synthetic construct
RAFSGLEGLEHLNLGGNAIR

SEQ ID NO: 37 - protein, 135 aa, synthetic construct
NLKELHISSDSFLCDCQLKWLPPWLIGRMLQAFVTATCAHPESLKGQSIFSVPPESFVCDDFLKPQIITQPETTMAMVGKDIRFTCSAASSSSSPMTFAWKKDNEVLTNADMENFVHVHAQDGEVMEYTTILHLR

SEQ ID NO: 38 - protein, 8 aa, synthetic construct
ATGNPPPR

SEQ ID NO: 39 - protein, 16 aa, synthetic construct
KLQRNNISKLTDGAFW

SEQ ID NO: 40 - protein, 45 aa, synthetic construct
SHKARLTVNVLPSFTKTPHDITIRTTTVARLECAATGHPNPQIAW

SEQ ID NO: 41 - protein, 7 aa, synthetic construct
LTDGAFW

SEQ ID NO: 42 - protein, 78 aa, synthetic construct
SVPPESFVCDDFLKPQIITQPETTMAMVGKDIRFTCSAASSSSSPMTFAWKKDNEVLTNADMENFVHVHAQDGEVMEY

SEQ ID NO: 43 - protein, 30 aa, synthetic construct; identical to SEQ ID NO: 26

SEQ ID NO: 44 - protein, 21 aa, synthetic construct
ARLTVNVLPSFTKTPHDITIR

SEQ ID NO: 45 - protein, 107 aa, synthetic construct
MLQAFVTATCAHPESLKGQSIFSVPPESFVCDDFLKPQIITQPETTMAMVGKDIRFTCSAASSSSSPMTFAWKKDNEVLTNADMENFVHVHAQDGEVMEYTTILHLR

SEQ ID NO: 46 - protein, 73 aa, synthetic construct
MLQAFVTATCAHPESLKGQSIFSVPPESFVCDDFLKPQIITQPETTMAMVGKDIRFTCSAASSSSSPMTFAWK

SEQ ID NO: 47 - protein, 48 aa, synthetic construct
SVPPESFVCDDFLKPQIITQPETTMAMVGKDIRFTCSAASSSSSPMTF

SEQ ID NO: 48 - protein, 19 aa, synthetic construct
AYLSLEVLDLSLNNITEVR

SEQ ID NO: 49 - protein, 28 aa, synthetic construct
VLDLDHNEISGTIEDTSGAFSGLDSLSK

SEQ ID NO: 50 - protein, 34 aa, synthetic construct
KDNEVLTNADMENFVHVHAQDGEVMEYTTILHLR

SEQ ID NO: 51 - protein, 31 aa, synthetic construct
DNEVLTNADMENFVHVHAQDGEVMEYTTILH

SEQ ID NO: 52 - protein, 33 aa, synthetic construct
DNEVLTNADMENFVHVHAQDGEVMEYTTILHLR

SEQ ID NO: 53 - protein, 39 aa, synthetic construct
IDDAGVYSCTAQNSAGSISANATLTVLETPSLVVPLEDR

SEQ ID NO: 54 - protein, 13 aa, synthetic construct
VVSVGETVALQCK

SEQ ID NO: 55 - protein, 22 aa, synthetic construct
SLNNITEVRNTCFPHGPPIKEL

SEQ ID NO: 56 - protein, 11 aa, synthetic construct
SFCQKLHELVL

SEQ ID NO: 57 - protein, 18 aa, synthetic construct
DLDHNEISGTIEDTSGAF

SEQ ID NO: 58 - protein, 15 aa, synthetic construct
HISSDSFLCDCQLKW

SEQ ID NO: 59 - protein, 14 aa, synthetic construct
QAFVTATCAHPESL

SEQ ID NO: 60 - protein, 11 aa, synthetic construct
VTATCAHPESL

SEQ ID NO: 61 - protein, 17 aa, synthetic construct
VTATCAHPESLKGQSIF

SEQ ID NO: 62 - protein, 25 aa, synthetic construct
SVPPESFVCDDFLKPQIITQPETTM

SEQ ID NO: 63 - protein, 21 aa, synthetic construct
AMVGKDIRFTCSAASSSSSPM

SEQ ID NO: 64 - protein, 7 aa, synthetic construct
HLRQVTF

SEQ ID NO: 65 - protein, 18 aa, synthetic construct
GHEGRYQCVITNHFGSTY

SEQ ID NO: 66 - protein, 14 aa, synthetic construct
ECAATGHPNPQIAW

SEQ ID NO: 67 - protein, 13 aa, synthetic construct
FITDVKIDDAGVY

SEQ ID NO: 68 - protein, 17 aa, synthetic construct
SCTAQNSAGSISANATL

SEQ ID NO: 69 - protein, 17 aa, synthetic construct
TCEMSNTLGTERAHSQL